European Patent Application EP 4 740 960 A1, published May 13, 2026. Title: 一种治疗含TP53基因突变肿瘤的药物. Applicant: 中国科学院分子细胞科学卓越创新中心. The sequence listing filed with the application follows.

SEQUENCE LISTING (98 sequences)

SEQ ID NO: 1 - RNA, 20 nt, Artificial sequence
  source 1..20: mol_type = other RNA
gctataaaactggaagttag

SEQ ID NO: 2 - RNA, 20 nt, Artificial sequence
  source 1..20: mol_type = other RNA
tgtatttcagaggctccaaa

SEQ ID NO: 3 - RNA, 20 nt, Artificial sequence
  source 1..20: mol_type = other RNA
acgaaatatggacgttcaag

SEQ ID NO: 4 - RNA, 20 nt, Artificial sequence
  source 1..20: mol_type = other RNA
tgggtcatccactgcccatt

SEQ ID NO: 5 - RNA, 20 nt, Artificial sequence
  source 1..20: mol_type = other RNA
tggcataaacccgggactaa

SEQ ID NO: 6 - RNA, 20 nt, Artificial sequence
  source 1..20: mol_type = other RNA
tttgacctacagcttgccca

SEQ ID NO: 7 - RNA, 20 nt, Artificial sequence
  source 1..20: mol_type = other RNA
gttgagagcgtggagttaag

SEQ ID NO: 8 - RNA, 20 nt, Artificial sequence
  source 1..20: mol_type = other RNA
tgaggtccagctgaaccata

SEQ ID NO: 9 - RNA, 20 nt, Artificial sequence
  source 1..20: mol_type = other RNA
gggcatcattaccctggacc

SEQ ID NO: 10 - RNA, 20 nt, Artificial sequence
  source 1..20: mol_type = other RNA
ctaccagggaagtatggtat

SEQ ID NO: 11 - RNA, 21 nt, Artificial sequence
  source 1..21: mol_type = other RNA
gaacgaaatatggacgttcaa

SEQ ID NO: 12 - RNA, 21 nt, Artificial sequence
  source 1..21: mol_type = other RNA
ttgaacgtccatatttcgttc

SEQ ID NO: 13 - RNA, 21 nt, Artificial sequence
  source 1..21: mol_type = other RNA
ggacttaagagatcagttgaa

SEQ ID NO: 14 - RNA, 21 nt, Artificial sequence
  source 1..21: mol_type = other RNA
ttcaactgatctcttaagtcc

SEQ ID NO: 15 - RNA, 21 nt, Artificial sequence
  source 1..21: mol_type = other RNA
ggttatgaggcagcatatggt

SEQ ID NO: 16 - RNA, 21 nt, Artificial sequence
  source 1..21: mol_type = other RNA
accatatgctgcctcataacc

SEQ ID NO: 17 - RNA, 19 nt, Artificial sequence
  source 1..19: mol_type = other RNA
cagctattcccttcagcaa

SEQ ID NO: 18 - RNA, 19 nt, Artificial sequence
  source 1..19: mol_type = other RNA
ttgctgaagggaatagctg

SEQ ID NO: 19 - RNA, 19 nt, Artificial sequence
  source 1..19: mol_type = other RNA
ccagaacaacagaaccaaa

SEQ ID NO: 20 - RNA, 19 nt, Artificial sequence
  source 1..19: mol_type = other RNA
tttggttctgttgttctgg

SEQ ID NO: 21 - RNA, 19 nt, Artificial sequence
  source 1..19: mol_type = other RNA
ggatgatcacactctacca

SEQ ID NO: 22 - RNA, 19 nt, Artificial sequence
  source 1..19: mol_type = other RNA
tggtagagtgtgatcatcc

SEQ ID NO: 23 - RNA, 19 nt, Artificial sequence
  source 1..19: mol_type = other RNA
gcaaagatctctccagtaa

SEQ ID NO: 24 - RNA, 19 nt, Artificial sequence
  source 1..19: mol_type = other RNA
ttactggagagatctttgc

SEQ ID NO: 25 - RNA, 21 nt, Artificial sequence
  source 1..21: mol_type = other RNA
gaaggaggacgtattctagta

SEQ ID NO: 26 - RNA, 21 nt, Artificial sequence
  source 1..21: mol_type = other RNA
tactagaatacgtcctccttc

SEQ ID NO: 27 - RNA, 19 nt, Artificial sequence
  source 1..19: mol_type = other RNA
gacgtattctagtacagaa

SEQ ID NO: 28 - RNA, 19 nt, Artificial sequence
  source 1..19: mol_type = other RNA
ttctgtactagaatacgtc

SEQ ID NO: 29 - RNA, 19 nt, Artificial sequence
  source 1..19: mol_type = other RNA
cacgaatagcagtgtttaa

SEQ ID NO: 30 - RNA, 19 nt, Artificial sequence
  source 1..19: mol_type = other RNA
ttaaacactgctattcgtg

SEQ ID NO: 31 - RNA, 19 nt, Artificial sequence
  source 1..19: mol_type = other RNA
gaaactctctgctatgtta

SEQ ID NO: 32 - RNA, 19 nt, Artificial sequence
  source 1..19: mol_type = other RNA
taacatagcagagagtttc

SEQ ID NO: 33 - RNA, 19 nt, Artificial sequence
  source 1..19: mol_type = other RNA
gacaaagttcattactaca

SEQ ID NO: 34 - RNA, 19 nt, Artificial sequence
  source 1..19: mol_type = other RNA
tgtagtaatgaactttgtc

SEQ ID NO: 35 - RNA, 21 nt, Artificial sequence
  source 1..21: mol_type = other RNA
gaaggacttaagagatcagtt

SEQ ID NO: 36 - RNA, 21 nt, Artificial sequence
  source 1..21: mol_type = other RNA
aactgatctcttaagtccttc

SEQ ID NO: 37 - RNA, 19 nt, Artificial sequence
  source 1..19: mol_type = other RNA
gacttaagagatcagttga

SEQ ID NO: 38 - RNA, 19 nt, Artificial sequence
  source 1..19: mol_type = other RNA
tcaactgatctcttaagtc

SEQ ID NO: 39 - RNA, 21 nt, Artificial sequence
  source 1..21: mol_type = other RNA
gaaaggcattgaacgaaatat

SEQ ID NO: 40 - RNA, 21 nt, Artificial sequence
  source 1..21: mol_type = other RNA
atatttcgttcaatgcctttc

SEQ ID NO: 41 - RNA, 19 nt, Artificial sequence
  source 1..19: mol_type = other RNA
ggacgttcaagaggtgcaa

SEQ ID NO: 42 - RNA, 19 nt, Artificial sequence
  source 1..19: mol_type = other RNA
ttgcacctcttgaacgtcc

SEQ ID NO: 43 - RNA, 19 nt, Artificial sequence
  source 1..19: mol_type = other RNA
gttcaagaggtgcaatata

SEQ ID NO: 44 - RNA, 19 nt, Artificial sequence
  source 1..19: mol_type = other RNA
tatattgcacctcttgaac

SEQ ID NO: 45 - RNA, 19 nt, Artificial sequence
  source 1..19: mol_type = other RNA
gcaatatacatttgaccta

SEQ ID NO: 46 - RNA, 19 nt, Artificial sequence
  source 1..19: mol_type = other RNA
taggtcaaatgtatattgc

SEQ ID NO: 47 - RNA, 19 nt, Artificial sequence
  source 1..19: mol_type = other RNA
ggtggtgcttacggagaaa

SEQ ID NO: 48 - RNA, 19 nt, Artificial sequence
  source 1..19: mol_type = other RNA
tttctccgtaagcaccacc

SEQ ID NO: 49 - RNA, 19 nt, Artificial sequence
  source 1..19: mol_type = other RNA
ggagttaagaggagaatca

SEQ ID NO: 50 - RNA, 19 nt, Artificial sequence
  source 1..19: mol_type = other RNA
tgattctcctcttaactcc

SEQ ID NO: 51 - RNA, 19 nt, Artificial sequence
  source 1..19: mol_type = other RNA
gaccaaattccttccttta

SEQ ID NO: 52 - RNA, 19 nt, Artificial sequence
  source 1..19: mol_type = other RNA
taaaggaaggaatttggtc

SEQ ID NO: 53 - RNA, 58 nt, Artificial sequence
  source 1..58: mol_type = other RNA
ccgggaacgaaatatggacgttcaactcgagttgaacgtccatatttcgttctttttg

SEQ ID NO: 54 - RNA, 58 nt, Artificial sequence
  source 1..58: mol_type = other RNA
aattcaaaaagaacgaaatatggacgttcaactcgagttgaacgtccatatttcgttc

SEQ ID NO: 55 - RNA, 58 nt, Artificial sequence
  source 1..58: mol_type = other RNA
ccggggacttaagagatcagttgaactcgagttcaactgatctcttaagtcctttttg

SEQ ID NO: 56 - RNA, 58 nt, Artificial sequence
  source 1..58: mol_type = other RNA
aattcaaaaaggacttaagagatcagttgaactcgagttcaactgatctcttaagtcc

SEQ ID NO: 57 - RNA, 58 nt, Artificial sequence
  source 1..58: mol_type = other RNA
ccggggttatgaggcagcatatggtctcgagaccatatgctgcctcataacctttttg

SEQ ID NO: 58 - RNA, 58 nt, Artificial sequence
  source 1..58: mol_type = other RNA
aattcaaaaaggttatgaggcagcatatggtctcgagaccatatgctgcctcataacc

SEQ ID NO: 59 - RNA, 54 nt, Artificial sequence
  source 1..54: mol_type = other RNA
ccggcagctattcccttcagcaactcgagttgctgaagggaatagctgtttttg

SEQ ID NO: 60 - RNA, 54 nt, Artificial sequence
  source 1..54: mol_type = other RNA
aattcaaaaacagctattcccttcagcaactcgagttgctgaagggaatagctg

SEQ ID NO: 61 - RNA, 54 nt, Artificial sequence
  source 1..54: mol_type = other RNA
ccggccagaacaacagaaccaaactcgagtttggttctgttgttctggtttttg

SEQ ID NO: 62 - RNA, 54 nt, Artificial sequence
  source 1..54: mol_type = other RNA
aattcaaaaaccagaacaacagaaccaaactcgagtttggttctgttgttctgg

SEQ ID NO: 63 - RNA, 54 nt, Artificial sequence
  source 1..54: mol_type = other RNA
ccggggatgatcacactctaccactcgagtggtagagtgtgatcatcctttttg

SEQ ID NO: 64 - RNA, 54 nt, Artificial sequence
  source 1..54: mol_type = other RNA
aattcaaaaaggatgatcacactctaccactcgagtggtagagtgtgatcatcc

SEQ ID NO: 65 - RNA, 54 nt, Artificial sequence
  source 1..54: mol_type = other RNA
ccgggcaaagatctctccagtaactcgagttactggagagatctttgctttttg

SEQ ID NO: 66 - RNA, 54 nt, Artificial sequence
  source 1..54: mol_type = other RNA
aattcaaaaagcaaagatctctccagtaactcgagttactggagagatctttgc

SEQ ID NO: 67 - RNA, 58 nt, Artificial sequence
  source 1..58: mol_type = other RNA
ccgggaaggaggacgtattctagtactcgagtactagaatacgtcctccttctttttg

SEQ ID NO: 68 - RNA, 58 nt, Artificial sequence
  source 1..58: mol_type = other RNA
aattcaaaaagaaggaggacgtattctagtactcgagtactagaatacgtcctccttc

SEQ ID NO: 69 - RNA, 54 nt, Artificial sequence
  source 1..54: mol_type = other RNA
ccgggacgtattctagtacagaactcgagttctgtactagaatacgtctttttg

SEQ ID NO: 70 - RNA, 54 nt, Artificial sequence
  source 1..54: mol_type = other RNA
aattcaaaaagacgtattctagtacagaactcgagttctgtactagaatacgtc

SEQ ID NO: 71 - RNA, 54 nt, Artificial sequence
  source 1..54: mol_type = other RNA
ccggcacgaatagcagtgtttaactcgagttaaacactgctattcgtgtttttg

SEQ ID NO: 72 - RNA, 54 nt, Artificial sequence
  source 1..54: mol_type = other RNA
aattcaaaaacacgaatagcagtgtttaactcgagttaaacactgctattcgtg

SEQ ID NO: 73 - RNA, 54 nt, Artificial sequence
  source 1..54: mol_type = other RNA
ccgggaaactctctgctatgttactcgagtaacatagcagagagtttctttttg

SEQ ID NO: 74 - RNA, 54 nt, Artificial sequence
  source 1..54: mol_type = other RNA
aattcaaaaagaaactctctgctatgttactcgagtaacatagcagagagtttc

SEQ ID NO: 75 - RNA, 54 nt, Artificial sequence
  source 1..54: mol_type = other RNA
ccgggacaaagttcattactacactcgagtgtagtaatgaactttgtctttttg

SEQ ID NO: 76 - RNA, 54 nt, Artificial sequence
  source 1..54: mol_type = other RNA
aattcaaaaagacaaagttcattactacactcgagtgtagtaatgaactttgtc

SEQ ID NO: 77 - RNA, 58 nt, Artificial sequence
  source 1..58: mol_type = other RNA
ccgggaaggacttaagagatcagttctcgagaactgatctcttaagtccttctttttg

SEQ ID NO: 78 - RNA, 58 nt, Artificial sequence
  source 1..58: mol_type = other RNA
aattcaaaaagaaggacttaagagatcagttctcgagaactgatctcttaagtccttc

SEQ ID NO: 79 - RNA, 54 nt, Artificial sequence
  source 1..54: mol_type = other RNA
ccgggacttaagagatcagttgactcgagtcaactgatctcttaagtctttttg

SEQ ID NO: 80 - RNA, 54 nt, Artificial sequence
  source 1..54: mol_type = other RNA
aattcaaaaagacttaagagatcagttgactcgagtcaactgatctcttaagtc

SEQ ID NO: 81 - RNA, 58 nt, Artificial sequence
  source 1..58: mol_type = other RNA
ccgggaaaggcattgaacgaaatatctcgagatatttcgttcaatgcctttctttttg

SEQ ID NO: 82 - RNA, 58 nt, Artificial sequence
  source 1..58: mol_type = other RNA
aattcaaaaagaaaggcattgaacgaaatatctcgagatatttcgttcaatgcctttc

SEQ ID NO: 83 - RNA, 54 nt, Artificial sequence
  source 1..54: mol_type = other RNA
ccggggacgttcaagaggtgcaactcgagttgcacctcttgaacgtcctttttg

SEQ ID NO: 84 - RNA, 54 nt, Artificial sequence
  source 1..54: mol_type = other RNA
aattcaaaaaggacgttcaagaggtgcaactcgagttgcacctcttgaacgtcc

SEQ ID NO: 85 - RNA, 54 nt, Artificial sequence
  source 1..54: mol_type = other RNA
ccgggttcaagaggtgcaatatactcgagtatattgcacctcttgaactttttg

SEQ ID NO: 86 - RNA, 54 nt, Artificial sequence
  source 1..54: mol_type = other RNA
aattcaaaaagttcaagaggtgcaatatactcgagtatattgcacctcttgaac

SEQ ID NO: 87 - RNA, 54 nt, Artificial sequence
  source 1..54: mol_type = other RNA
ccgggcaatatacatttgacctactcgagtaggtcaaatgtatattgctttttg

SEQ ID NO: 88 - RNA, 54 nt, Artificial sequence
  source 1..54: mol_type = other RNA
aattcaaaaagcaatatacatttgacctactcgagtaggtcaaatgtatattgc

SEQ ID NO: 89 - RNA, 54 nt, Artificial sequence
  source 1..54: mol_type = other RNA
ccggggtggtgcttacggagaaactcgagtttctccgtaagcaccacctttttg

SEQ ID NO: 90 - RNA, 54 nt, Artificial sequence
  source 1..54: mol_type = other RNA
aattcaaaaaggtggtgcttacggagaaactcgagtttctccgtaagcaccacc

SEQ ID NO: 91 - RNA, 54 nt, Artificial sequence
  source 1..54: mol_type = other RNA
ccggggagttaagaggagaatcactcgagtgattctcctcttaactcctttttg

SEQ ID NO: 92 - RNA, 54 nt, Artificial sequence
  source 1..54: mol_type = other RNA
aattcaaaaaggagttaagaggagaatcactcgagtgattctcctcttaactcc

SEQ ID NO: 93 - RNA, 54 nt, Artificial sequence
  source 1..54: mol_type = other RNA
ccgggaccaaattccttcctttactcgagtaaaggaaggaatttggtctttttg

SEQ ID NO: 94 - RNA, 54 nt, Artificial sequence
  source 1..54: mol_type = other RNA
aattcaaaaagaccaaattccttcctttactcgagtaaaggaaggaatttggtc

SEQ ID NO: 95 - RNA, 20 nt, Artificial sequence
  source 1..20: mol_type = other RNA
agtgaagccctccgagtgtc

SEQ ID NO: 96 - RNA, 20 nt, Artificial sequence
  source 1..20: mol_type = other RNA
gaccctgtcaccgagacccc

SEQ ID NO: 97 - RNA, 20 nt, Artificial sequence
  source 1..20: mol_type = other RNA
ttctagattggcattaaccc

SEQ ID NO: 98 - RNA, 20 nt, Artificial sequence
  source 1..20: mol_type = other RNA
ccgggaaggagggcgcatcc